European Patent Application EP 4 335 918 A2, published March 13, 2024. Title: Composition and Methods of Genome Editing of B-Cells. Applicant: Dana-Farber Cancer Institute, Inc. Application EP. The sequence listing filed with the application follows.

SEQUENCE LISTING (12 sequences)

SEQ ID NO: 1 - protein, 9 aa, synthetic construct
  REGION 1..9: note = Synthetic Polypeptide
LAGLIDADG

SEQ ID NO: 2 - protein, 6 aa, synthetic construct
  REGION 1..6: note = Synthetic Polypeptide
GIYYIG

SEQ ID NO: 3 - protein, 5 aa, synthetic construct
  REGION 1..5: note = Synthetic Polypeptide
TGEKP

SEQ ID NO: 4 - protein, 6 aa, synthetic construct
  REGION 1..6: note = Synthetic Polypeptide
TGGQRP

SEQ ID NO: 5 - protein, 5 aa, synthetic construct
  REGION 1..5: note = Synthetic Polypeptide
TGQKP

SEQ ID NO: 6 - protein, 6 aa, synthetic construct
  REGION 1..6: note = Synthetic Polypeptide
TGSQKP

SEQ ID NO: 7 - DNA, 20 bp, synthetic construct
  misc_feature 1..20: note = Synthetic Polynucleotide
  source 1..20: mol_type = other DNA
tgaacagagagaactcacca

SEQ ID NO: 8 - DNA, 20 bp, synthetic construct
  misc_feature 1..20: note = Synthetic Polynucleotide
  source 1..20: mol_type = other DNA
gcattgcaggttggtcctcg

SEQ ID NO: 9 - DNA, 20 bp, synthetic construct
  misc_feature 1..20: note = Synthetic Polynucleotide
  source 1..20: mol_type = other DNA
ttaggacccagagggaacca

SEQ ID NO: 10 - DNA, 20 bp, synthetic construct
  misc_feature 1..20: note = Synthetic Polynucleotide
  source 1..20: mol_type = other DNA
gggcatttaagatttgccat

SEQ ID NO: 11 - DNA, 1359 bp, synthetic construct
  misc_feature 1..1359: note = Synthetic Polynucleotide
  source 1..1359: mol_type = other DNA
atggaagtgcagctggtggaaagcggcggaggcctggtgcagcctggcagatctctgagactgagctgtgccgccagcggcttcaccttcgacgactacgccatgcactgggtgcgccaggcccctggaaaaggcctggaatgggtgtccgccatcacctggaacagcggccacatcgattacgccgacagcgtggaaggccggttcaccatcagccgggacaacgccaagaacagcctgtacctgcagatgaactccctgcgggccgaggacaccgccgtgtactactgtgccaaagtttcctacctgagcaccgccagcagcctggattattggggccagggcacactcgtgaccgtgtcctcggcctccaccaagggcccatcggtcttccccctggcaccctcctccaagagcacctctgggggcacagcagccctgggctgcctggtcaaggactacttccccgaaccggtgacggtgtcgtggaactcaggcgccctgaccagcggcgtgcacaccttcccggctgtcctacagtcctcaggactctactccctcagcagcgtggtgaccgtgccctccagcagcttgggcacccagacctacatctgcaacgtgaatcacaagcccagcaacaccaaggtggacaagaaagttgagcccaaatcttgtgacaaaactcacacatgcccaccgtgcccagcacctgaactcctggggggaccgtcagtcttcctcttccccccaaaacccaaggacaccctcatgatctcccggacccctgaggtcacatgcgtggtggtggacgtgagccacgaagaccctgaggtcaagttcaactggtacgtggacggcgtggaggtgcataatgccaagacaaagccgcgggaggagcagtacaacagcacgtaccgtgtggtcagcgtcctcaccgtcctgcaccaggactggctgaatggcaaggagtacaagtgcaaggtctccaacaaagccctcccagcccccatcgagaaaaccatctccaaagccaaagggcagccccgagaaccacaggtgtacaccctgcccccatcccgggatgagctgaccaagaaccaggtcagcctgacctgcctggtcaaaggcttctatcccagcgacatcgccgtggagtgggagagcaatgggcagccggagaacaactacaagaccacgcctcccgtgctggactccgacggctccttcttcctctacagcaagctcaccgtggacaagagcaggtggcagcaggggaacgtcttctcatgctccgtgatgcatgaggctctgcacaaccactacacacagaagagcctctccctgtctccgggtaaatga

SEQ ID NO: 12 - DNA, 648 bp, synthetic construct
  misc_feature 1..648: note = Synthetic Polynucleotide
  source 1..648: mol_type = other DNA
atggacatccagatgacccagagccccagcagcctgtctgccagcgtgggcgacagagtgaccatcacctgtagagccagccagggcatccggaactacctggcctggtatcagcagaagcccggcaaggcccccaagctgctgatctacgccgccagcacactgcagagcggcgtgccaagcagattttccggcagcggctccggcaccgacttcaccctgacaatcagctccctgcagcccgaggacgtggccacctactactgccagcggtacaacagagccccctacacctttggccagggcaccaaggtggaaatcaagggaactgtggctgcaccatctgtcttcatcttcccgccatctgatgagcagttgaaatctggaactgcctctgttgtgtgcctgctgaataacttctatcccagagaggccaaagtacagtggaaggtggataacgccctccaatcgggtaactcccaggagagtgtcacagagcaggacagcaaggacagcacctacagcctcagcagcaccctgacgctgagcaaagcagactacgagaaacacaaagtctacgcctgcgaagtcacccatcagggcctgagctcgcccgtcacaaagagcttcaacaggggagagtgttag